European Patent Application EP 4 751 723 A2, published June 3, 2026. Title: Use of telomerase inhibitors for the treatment of myeloproliferative disorders and myeloproliferative neoplasms. Applicant: Geron Corporation. Application EP. The sequence listing filed with the application follows.

SEQUENCE LISTING (23 sequences)

SEQ ID NO: 1 - RNA, 554 nt, Homo sapiens
  source 1..554: mol_type = other RNA
gggttgcggagggtgggcctgggaggggtggtggccattttttgtctaaccctaactgagaagggcgtaggcgccgtgcttttgctccccgcgcgctgtttttctcgctgactttcagcgggcggaaaagcctcggcctgccgccttccaccgttcattctagagcaaacaaaaaatgtcagctgctggcccgttcgcctcccggggacctgcggcgggtcgcctgcccagcccccgaaccccgcctggagccgcggtcggcccggggcttctccggaggcacccactgccaccgcgaagagttgggctctgtcagccgcgggtctctcgggggcgagggcgaggttcaccgtttcaggccgcaggaagaggaacggagcgagtcccgccgcggcgcgattccctgagctgtgggacgtgcacccaggactcggctcacacatgcagttcgctttcctgttggtggggggaacgccgatcgtgcgcatccgtcacccctcgccggcagtgggggcttgtgaacccccaaacctgactgactgggccagtgtgct

SEQ ID NO: 2 - DNA, 20 bp, Homo sapiens
  source 1..20: mol_type = genomic DNA
acattttttgtttgctctag

SEQ ID NO: 3 - DNA, 30 bp, Homo sapiens
  source 1..30: mol_type = genomic DNA
gctctagaatgaacggtggaaggcggcagg

SEQ ID NO: 4 - DNA, 14 bp, Homo sapiens
  source 1..14: mol_type = genomic DNA
gtggaggcggcagg

SEQ ID NO: 5 - DNA, 13 bp, Homo sapiens
  source 1..13: mol_type = genomic DNA
ggaaggcggcagg

SEQ ID NO: 6 - DNA, 13 bp, Homo sapiens
  source 1..13: mol_type = genomic DNA
gtggaaggcggca

SEQ ID NO: 7 - DNA, 11 bp, Homo sapiens
  source 1..11: mol_type = genomic DNA
gtggaaggcgg

SEQ ID NO: 8 - DNA, 13 bp, Homo sapiens
  source 1..13: mol_type = genomic DNA
cggtggaaggcgg

SEQ ID NO: 9 - DNA, 13 bp, Homo sapiens
  source 1..13: mol_type = genomic DNA
acggtggaaggcg

SEQ ID NO: 10 - DNA, 16 bp, Homo sapiens
  source 1..16: mol_type = genomic DNA
aacggtggaaggcggc

SEQ ID NO: 11 - DNA, 18 bp, Homo sapiens
  source 1..18: mol_type = genomic DNA
atgaacggtggaaggcgg

SEQ ID NO: 12 - DNA, 13 bp, Homo sapiens
  source 1..13: mol_type = genomic DNA
tagggttagacaa

SEQ ID NO: 13 - DNA, 13 bp, Homo sapiens
  source 1..13: mol_type = genomic DNA
cagttagggttag

SEQ ID NO: 14 - DNA, 12 bp, Homo sapiens
  source 1..12: mol_type = genomic DNA
tagggttagaca

SEQ ID NO: 15 - DNA, 11 bp, Homo sapiens
  source 1..11: mol_type = genomic DNA
tagggttagac

SEQ ID NO: 16 - DNA, 11 bp, Homo sapiens
  source 1..11: mol_type = genomic DNA
gttagggttag

SEQ ID NO: 17 - DNA, 13 bp, Homo sapiens
  source 1..13: mol_type = genomic DNA
gttagggttagac

SEQ ID NO: 18 - DNA, 15 bp, Homo sapiens
  source 1..15: mol_type = genomic DNA
gttagggttagacaa

SEQ ID NO: 19-20 - skipped (2 entries)

SEQ ID NO: 21 - DNA, 12 bp, Homo sapiens
  source 1..12: mol_type = genomic DNA
cccttctcagtt

SEQ ID NO: 22 - DNA, 12 bp, Homo sapiens
  source 1..12: mol_type = genomic DNA
cgcccttctcag

SEQ ID NO: 23 - RNA, 11 nt, synthetic construct
  misc_feature 1..11: note = hTR template inhibitor
  source 1..11: mol_type = other RNA
ctaaccctaac